European Patent Specification EP 3 758 744 B1, published May 8, 2024. Title: Polypepetide and Vaccine. Applicant: One Health Ventures Ltd. The sequence listing filed with the application follows.

SEQUENCE LISTING (68 sequences)

SEQ ID NO: 1 - protein, 26 aa, Artificial Sequence
  Protein fragment
VYVGKALLTNDTQQEQKLKSQSFTCK

SEQ ID NO: 2 - protein, 24 aa, Artificial Sequence
  Protein fragment
THNVPSQDILVPANTTVEVIAYLK

SEQ ID NO: 3 - protein, 47 aa, Artificial Sequence
  Protein fragment
DELIVKVRNLNTNNVQEYVIPVDKKEKSNDSNIVKYRSLYIKAPGIK

SEQ ID NO: 4 - protein, 10 aa, Artificial Sequence
  Protein fragment mutant
  Xaa (6)..(6): any amino acid other than Tyr, or is a deletion
RMEKYXPNAM

SEQ ID NO: 5 - protein, 10 aa, Artificial Sequence
  Protein fragment mutant
  Xaa (6)..(6): any amino acid other than Tyr, or is a deletion
GEIPSXLAFP

SEQ ID NO: 6 - protein, 10 aa, Artificial Sequence
  Protein fragment mutant
  Xaa (6)..(6): any amino acid other than His, or is a deletion
SKEITXNVPS

SEQ ID NO: 7 - protein, 10 aa, Artificial Sequence
  Protein fragment mutant
  Xaa (6)..(6): any amino acid other than Val, or is a deletion
LEDVYXGKAL

SEQ ID NO: 8 - protein, 10 aa, Artificial Sequence
  Protein fragment mutant
  Xaa (6)..(6): any amino acid other than Phe, or is a deletion
LKSQSXTCKN

SEQ ID NO: 9 - protein, 10 aa, Artificial Sequence
  Protein fragment mutant
  Xaa (6)..(6): any amino acid other than Val, or is a deletion
NTTVEXIAYL

SEQ ID NO: 10 - protein, 10 aa, Artificial Sequence
  Protein fragment mutant
  Xaa (6)..(6): any amino acid other than Ala, or is a deletion
TVEVIXYLKK

SEQ ID NO: 11 - protein, 328 aa, Clostridium perfringens
MKKNLVKSLAIASAVISIYSIVNIVSPTNVIAKEISNTVSNEMSKKASYDNVDTLIEKGRYNTKYNYLKRMEKYYPNAMAYFDKVTINPQGNDFYINNPKVELDGEPSMNYLEDVYVGKALLTNDTQQEQKLKSQSFTCKNTDTVTATTTHTVGTSIQATAKFTVPFNETGVSLTTSYSFANTNTNTNSKEITHNVPSQDILVPANTTVEVIAYLKKVNVKGNVKLVGQVSGSEWGEIPSYLAFPRDGYKFSLSDTVNKSDLNEDGTININGKGNYSAVMGDELIVKVRNLNTNNVQEYVIPVDKKEKSNDSNIVKYRSLSIKAPGIK

SEQ ID NO: 12 - protein, 296 aa, Artificial Sequence
  Construct for crystal structure analysis
KEISNTVSNEMSKKASYDNVDTLIEKGRYNTKYNYLKRMEKYYPNAMAYFDKVTINPQGNDFYINNPKVELDGEPSMNYLEDVYVGKALLTNDTQQEQKLKSQSFTCKNTDTVTATTTHTVGTSIQATAKFTVPFNETGVSLTTSYSFANTNTNTNSKEITHNVPSQDILVPANTTVEVIAYLKKVNVKGNVKLVGQVSGSEWGEIPSYLAFPRDGYKFSLSDTVNKSDLNEDGTININGKGNYSAVMGDELIVKVRNLNTNNVQEYVIPVDKKEKSNDSNIVKYRSLSIKAPGIK

SEQ ID NO: 13 - protein, 263 aa, Clostridium perfringens
MGKASYDNVDTLIEKGRYNTKYNYLKRMEKYYPNAMAYFDKVTINPQGNDFYINNPKVELDGEPSMNYLEDVYVGKALLTNDTQQEQKLKSQSFTCKNTDTVTATTTHTVGTSIQATAKFTVPFNETGVSLTTSYSFANTNTNTNSKEITHNVPSQDILVPANTTVEVIAYLKKVNVKGNVKLVGQVSGSEWGEIPSYLAFPRDGYKFSLSDTVNKSDLNEDGTININGKGNYSAVMGDELIVKVRNLNTNNVQEYVIPVDKK

SEQ ID NO: 14 - protein, 263 aa, Artificial Sequence
  Mutant polypeptide
MGKASYDNVDTLIEKGRYNTKYNYLKRMEKYYPNAMAYFDKVTINPQGNDFYINNPKVELDGEPSMNYLEDVYVGKALLTNDTQQEQKLKSQSFTCKNTDTVTATTTHTVGTSIQATAKFTVPFNETGVSLTTSYSFANTNTNTNSKEITANVPSQDILVPANTTVEVIAYLKKVNVKGNVKLVGQVSGSEWGEIPSYLAFPRDGYKFSLSDTVNKSDLNEDGTININGKGNYSAVMGDELIVKVRNLNTNNVQEYVIPVDKK

SEQ ID NO: 15 - protein, 315 aa, Artificial Sequence
  Recombinant polypeptide
MKYLLPTAAAGLLLLAAQPAMAMGKASYDNVDTLIEKGRYNTKYNYLKRMEKYYPNAMAYFDKVTINPQGNDFYINNPKVELDGEPSMNYLEDVYVGKALLTNDTQQEQKLKSQSFTCKNTDTVTATTTHTVGTSIQATAKFTVPFNETGVSLTTSYSFANTNTNTNSKEITHNVPSQDILVPANTTVEVIAYLKKVNVKGNVKLVGQVSGSEWGEIPSYLAFPRDGYKFSLSDTVNKSDLNEDGTININGKGNYSAVMGDELIVKVRNLNTNNVQEYVIPVDKKEKSNDSNIVKYRSLYIKAPGIKLEHHHHHH

SEQ ID NO: 16 - protein, 263 aa, Artificial Sequence
  Mutant polypeptide
MGKASYDNVDTLIEKGRYNTKYNYLKRMEKYAPNAMAYFDKVTINPQGNDFYINNPKVELDGEPSMNYLEDVYVGKALLTNDTQQEQKLKSQSFTCKNTDTVTATTTHTVGTSIQATAKFTVPFNETGVSLTTSYSFANTNTNTNSKEITHNVPSQDILVPANTTVEVIAYLKKVNVKGNVKLVGQVSGSEWGEIPSALAFPRDGYKFSLSDTVNKSDLNEDGTININGKGNYSAVMGDELIVKVRNLNTNNVQEYVIPVDKK

SEQ ID NO: 17 - protein, 263 aa, Artificial Sequence
  Mutant polypeptide
MGKASYDNVDTLIEKGRYNTKYNYLKRMEKYAPNAMAYFDKVTINPQGNDFYINNPKVELDGEPSMNYLEDVYVGKALLTNDTQQEQKLKSQSFTCKNTDTVTATTTHTVGTSIQATAKFTVPFNETGVSLTTSYSFANTNTNTNSKEITANVPSQDILVPANTTVEVIAYLKKVNVKGNVKLVGQVSGSEWGEIPSALAFPRDGYKFSLSDTVNKSDLNEDGTININGKGNYSAVMGDELIVKVRNLNTNNVQEYVIPVDKK

SEQ ID NO: 18 - protein, 263 aa, Artificial Sequence
  Mutant polypeptide
MGKASYDNVDTLIEKGRYNTKYNYLKRMEKYAPNAMAYFDKVTINPQGNDFYINNPKVELDGEPSMNYLEDVYFGKALLTNDTQQEQKLKSQSFTCKNTDTVTATTTHTVGTSIQATAKFTVPFNETGVSLTTSYSFANTNTNTNSKEITHNVPSQDILVPANTTVEVIAYLKKVNVKGNVKLVGQVSGSEWGEIPSALAFPRDGYKFSLSDTVNKSDLNEDGTININGKGNYSAVMGDELIVKVRNLNTNNVQEYVIPVDKK

SEQ ID NO: 19 - protein, 263 aa, Artificial Sequence
  Mutant polypeptide
MGKASYDNVDTLIEKGRYNTKYNYLKRMEKYAPNAMAYFDKVTINPQGNDFYINNPKVELDGEPSMNYLEDVYVGKALLTNDTQQEQKLKSQSATCKNTDTVTATTTHTVGTSIQATAKFTVPFNETGVSLTTSYSFANTNTNTNSKEITHNVPSQDILVPANTTVEVIAYLKKVNVKGNVKLVGQVSGSEWGEIPSALAFPRDGYKFSLSDTVNKSDLNEDGTININGKGNYSAVMGDELIVKVRNLNTNNVQEYVIPVDKK

SEQ ID NO: 20 - protein, 263 aa, Artificial Sequence
  Mutant polypeptide
MGKASYDNVDTLIEKGRYNTKYNYLKRMEKYAPNAMAYFDKVTINPQGNDFYINNPKVELDGEPSMNYLEDVYVGKALLTNDTQQEQKLKSQSFTCKNTDTVTATTTHTVGTSIQATAKFTVPFNETGVSLTTSYSFANTNTNTNSKEITHNVPSQDILVPANTTVEAIAYLKKVNVKGNVKLVGQVSGSEWGEIPSALAFPRDGYKFSLSDTVNKSDLNEDGTININGKGNYSAVMGDELIVKVRNLNTNNVQEYVIPVDKK

SEQ ID NO: 21 - protein, 263 aa, Artificial Sequence
  Mutant polypeptide
MGKASYDNVDTLIEKGRYNTKYNYLKRMEKYAPNAMAYFDKVTINPQGNDFYINNPKVELDGEPSMNYLEDVYVGKALLTNDTQQEQKLKSQSFTCKNTDTVTATTTHTVGTSIQATAKFTVPFNETGVSLTTSYSFANTNTNTNSKEITHNVPSQDILVPANTTVEVIFYLKKVNVKGNVKLVGQVSGSEWGEIPSALAFPRDGYKFSLSDTVNKSDLNEDGTININGKGNYSAVMGDELIVKVRNLNTNNVQEYVIPVDKK

SEQ ID NO: 22 - protein, 263 aa, Artificial Sequence
  Mutant polypeptide
MGKASYDNVDTLIEKGRYNTKYNYLKRMEKYAPNAMAYFDKVTINPQGNDFYINNPKVELDGEPSMNYLEDVYFGKALLTNDTQQEQKLKSQSFTCKNTDTVTATTTHTVGTSIQATAKFTVPFNETGVSLTTSYSFANTNTNTNSKEITANVPSQDILVPANTTVEVIAYLKKVNVKGNVKLVGQVSGSEWGEIPSALAFPRDGYKFSLSDTVNKSDLNEDGTININGKGNYSAVMGDELIVKVRNLNTNNVQEYVIPVDKK

SEQ ID NO: 23 - protein, 263 aa, Artificial Sequence
  Mutant polypeptide
MGKASYDNVDTLIEKGRYNTKYNYLKRMEKYAPNAMAYFDKVTINPQGNDFYINNPKVELDGEPSMNYLEDVYVGKALLTNDTQQEQKLKSQSATCKNTDTVTATTTHTVGTSIQATAKFTVPFNETGVSLTTSYSFANTNTNTNSKEITANVPSQDILVPANTTVEVIAYLKKVNVKGNVKLVGQVSGSEWGEIPSALAFPRDGYKFSLSDTVNKSDLNEDGTININGKGNYSAVMGDELIVKVRNLNTNNVQEYVIPVDKK

SEQ ID NO: 24 - protein, 263 aa, Artificial Sequence
  Mutant polypeptide
MGKASYDNVDTLIEKGRYNTKYNYLKRMEKYAPNAMAYFDKVTINPQGNDFYINNPKVELDGEPSMNYLEDVYVGKALLTNDTQQEQKLKSQSFTCKNTDTVTATTTHTVGTSIQATAKFTVPFNETGVSLTTSYSFANTNTNTNSKEITANVPSQDILVPANTTVEAIAYLKKVNVKGNVKLVGQVSGSEWGEIPSALAFPRDGYKFSLSDTVNKSDLNEDGTININGKGNYSAVMGDELIVKVRNLNTNNVQEYVIPVDKK

SEQ ID NO: 25 - protein, 263 aa, Artificial Sequence
  Mutant polypeptide
MGKASYDNVDTLIEKGRYNTKYNYLKRMEKYAPNAMAYFDKVTINPQGNDFYINNPKVELDGEPSMNYLEDVYVGKALLTNDTQQEQKLKSQSFTCKNTDTVTATTTHTVGTSIQATAKFTVPFNETGVSLTTSYSFANTNTNTNSKEITANVPSQDILVPANTTVEVIFYLKKVNVKGNVKLVGQVSGSEWGEIPSALAFPRDGYKFSLSDTVNKSDLNEDGTININGKGNYSAVMGDELIVKVRNLNTNNVQEYVIPVDKK

SEQ ID NO: 26 - protein, 263 aa, Artificial Sequence
  Mutant polypeptide
MGKASYDNVDTLIEKGRYNTKYNYLKRMEKYAPNAMAYFDKVTINPQGNDFYINNPKVELDGEPSMNYLEDVYFGKALLTNDTQQEQKLKSQSATCKNTDTVTATTTHTVGTSIQATAKFTVPFNETGVSLTTSYSFANTNTNTNSKEITHNVPSQDILVPANTTVEVIAYLKKVNVKGNVKLVGQVSGSEWGEIPSALAFPRDGYKFSLSDTVNKSDLNEDGTININGKGNYSAVMGDELIVKVRNLNTNNVQEYVIPVDKK

SEQ ID NO: 27 - protein, 263 aa, Artificial Sequence
  Mutant polypeptide
MGKASYDNVDTLIEKGRYNTKYNYLKRMEKYAPNAMAYFDKVTINPQGNDFYINNPKVELDGEPSMNYLEDVYFGKALLTNDTQQEQKLKSQSFTCKNTDTVTATTTHTVGTSIQATAKFTVPFNETGVSLTTSYSFANTNTNTNSKEITHNVPSQDILVPANTTVEAIAYLKKVNVKGNVKLVGQVSGSEWGEIPSALAFPRDGYKFSLSDTVNKSDLNEDGTININGKGNYSAVMGDELIVKVRNLNTNNVQEYVIPVDKK

SEQ ID NO: 28 - protein, 263 aa, Artificial Sequence
  Mutant polypeptide
MGKASYDNVDTLIEKGRYNTKYNYLKRMEKYAPNAMAYFDKVTINPQGNDFYINNPKVELDGEPSMNYLEDVYFGKALLTNDTQQEQKLKSQSFTCKNTDTVTATTTHTVGTSIQATAKFTVPFNETGVSLTTSYSFANTNTNTNSKEITHNVPSQDILVPANTTVEVIFYLKKVNVKGNVKLVGQVSGSEWGEIPSALAFPRDGYKFSLSDTVNKSDLNEDGTININGKGNYSAVMGDELIVKVRNLNTNNVQEYVIPVDKK

SEQ ID NO: 29 - protein, 263 aa, Artificial Sequence
  Mutant polypeptide
MGKASYDNVDTLIEKGRYNTKYNYLKRMEKYAPNAMAYFDKVTINPQGNDFYINNPKVELDGEPSMNYLEDVYVGKALLTNDTQQEQKLKSQSATCKNTDTVTATTTHTVGTSIQATAKFTVPFNETGVSLTTSYSFANTNTNTNSKEITHNVPSQDILVPANTTVEAIAYLKKVNVKGNVKLVGQVSGSEWGEIPSALAFPRDGYKFSLSDTVNKSDLNEDGTININGKGNYSAVMGDELIVKVRNLNTNNVQEYVIPVDKK

SEQ ID NO: 30 - protein, 263 aa, Artificial Sequence
  Mutant polypeptide
MGKASYDNVDTLIEKGRYNTKYNYLKRMEKYAPNAMAYFDKVTINPQGNDFYINNPKVELDGEPSMNYLEDVYVGKALLTNDTQQEQKLKSQSATCKNTDTVTATTTHTVGTSIQATAKFTVPFNETGVSLTTSYSFANTNTNTNSKEITHNVPSQDILVPANTTVEVIFYLKKVNVKGNVKLVGQVSGSEWGEIPSALAFPRDGYKFSLSDTVNKSDLNEDGTININGKGNYSAVMGDELIVKVRNLNTNNVQEYVIPVDKK

SEQ ID NO: 31 - protein, 263 aa, Artificial Sequence
  Mutant polypeptide
MGKASYDNVDTLIEKGRYNTKYNYLKRMEKYAPNAMAYFDKVTINPQGNDFYINNPKVELDGEPSMNYLEDVYVGKALLTNDTQQEQKLKSQSFTCKNTDTVTATTTHTVGTSIQATAKFTVPFNETGVSLTTSYSFANTNTNTNSKEITHNVPSQDILVPANTTVEAIFYLKKVNVKGNVKLVGQVSGSEWGEIPSALAFPRDGYKFSLSDTVNKSDLNEDGTININGKGNYSAVMGDELIVKVRNLNTNNVQEYVIPVDKK

SEQ ID NO: 32 - protein, 263 aa, Artificial Sequence
  Mutant polypeptide
MGKASYDNVDTLIEKGRYNTKYNYLKRMEKYAPNAMAYFDKVTINPQGNDFYINNPKVELDGEPSMNYLEDVYFGKALLTNDTQQEQKLKSQSATCKNTDTVTATTTHTVGTSIQATAKFTVPFNETGVSLTTSYSFANTNTNTNSKEITANVPSQDILVPANTTVEVIAYLKKVNVKGNVKLVGQVSGSEWGEIPSALAFPRDGYKFSLSDTVNKSDLNEDGTININGKGNYSAVMGDELIVKVRNLNTNNVQEYVIPVDKK

SEQ ID NO: 33 - protein, 263 aa, Artificial Sequence
  Mutant polypeptide
MGKASYDNVDTLIEKGRYNTKYNYLKRMEKYAPNAMAYFDKVTINPQGNDFYINNPKVELDGEPSMNYLEDVYFGKALLTNDTQQEQKLKSQSFTCKNTDTVTATTTHTVGTSIQATAKFTVPFNETGVSLTTSYSFANTNTNTNSKEITANVPSQDILVPANTTVEAIAYLKKVNVKGNVKLVGQVSGSEWGEIPSALAFPRDGYKFSLSDTVNKSDLNEDGTININGKGNYSAVMGDELIVKVRNLNTNNVQEYVIPVDKK

SEQ ID NO: 34 - protein, 263 aa, Artificial Sequence
  Mutant polypeptide
MGKASYDNVDTLIEKGRYNTKYNYLKRMEKYAPNAMAYFDKVTINPQGNDFYINNPKVELDGEPSMNYLEDVYFGKALLTNDTQQEQKLKSQSFTCKNTDTVTATTTHTVGTSIQATAKFTVPFNETGVSLTTSYSFANTNTNTNSKEITANVPSQDILVPANTTVEVIFYLKKVNVKGNVKLVGQVSGSEWGEIPSALAFPRDGYKFSLSDTVNKSDLNEDGTININGKGNYSAVMGDELIVKVRNLNTNNVQEYVIPVDKK

SEQ ID NO: 35 - protein, 263 aa, Artificial Sequence
  Mutant polypeptide
MGKASYDNVDTLIEKGRYNTKYNYLKRMEKYAPNAMAYFDKVTINPQGNDFYINNPKVELDGEPSMNYLEDVYVGKALLTNDTQQEQKLKSQSATCKNTDTVTATTTHTVGTSIQATAKFTVPFNETGVSLTTSYSFANTNTNTNSKEITANVPSQDILVPANTTVEAIAYLKKVNVKGNVKLVGQVSGSEWGEIPSALAFPRDGYKFSLSDTVNKSDLNEDGTININGKGNYSAVMGDELIVKVRNLNTNNVQEYVIPVDKK

SEQ ID NO: 36 - protein, 263 aa, Artificial Sequence
  Mutant polypeptide
MGKASYDNVDTLIEKGRYNTKYNYLKRMEKYAPNAMAYFDKVTINPQGNDFYINNPKVELDGEPSMNYLEDVYVGKALLTNDTQQEQKLKSQSATCKNTDTVTATTTHTVGTSIQATAKFTVPFNETGVSLTTSYSFANTNTNTNSKEITANVPSQDILVPANTTVEVIFYLKKVNVKGNVKLVGQVSGSEWGEIPSALAFPRDGYKFSLSDTVNKSDLNEDGTININGKGNYSAVMGDELIVKVRNLNTNNVQEYVIPVDKK

SEQ ID NO: 37 - protein, 263 aa, Artificial Sequence
  Mutant polypeptide
MGKASYDNVDTLIEKGRYNTKYNYLKRMEKYAPNAMAYFDKVTINPQGNDFYINNPKVELDGEPSMNYLEDVYVGKALLTNDTQQEQKLKSQSFTCKNTDTVTATTTHTVGTSIQATAKFTVPFNETGVSLTTSYSFANTNTNTNSKEITANVPSQDILVPANTTVEAIFYLKKVNVKGNVKLVGQVSGSEWGEIPSALAFPRDGYKFSLSDTVNKSDLNEDGTININGKGNYSAVMGDELIVKVRNLNTNNVQEYVIPVDKK

SEQ ID NO: 38 - protein, 263 aa, Artificial Sequence
  Mutant polypeptide
MGKASYDNVDTLIEKGRYNTKYNYLKRMEKYAPNAMAYFDKVTINPQGNDFYINNPKVELDGEPSMNYLEDVYFGKALLTNDTQQEQKLKSQSATCKNTDTVTATTTHTVGTSIQATAKFTVPFNETGVSLTTSYSFANTNTNTNSKEITHNVPSQDILVPANTTVEAIAYLKKVNVKGNVKLVGQVSGSEWGEIPSALAFPRDGYKFSLSDTVNKSDLNEDGTININGKGNYSAVMGDELIVKVRNLNTNNVQEYVIPVDKK

SEQ ID NO: 39 - protein, 263 aa, Artificial Sequence
  Mutant polypeptide
MGKASYDNVDTLIEKGRYNTKYNYLKRMEKYAPNAMAYFDKVTINPQGNDFYINNPKVELDGEPSMNYLEDVYFGKALLTNDTQQEQKLKSQSATCKNTDTVTATTTHTVGTSIQATAKFTVPFNETGVSLTTSYSFANTNTNTNSKEITHNVPSQDILVPANTTVEVIFYLKKVNVKGNVKLVGQVSGSEWGEIPSALAFPRDGYKFSLSDTVNKSDLNEDGTININGKGNYSAVMGDELIVKVRNLNTNNVQEYVIPVDKK

SEQ ID NO: 40 - protein, 263 aa, Artificial Sequence
  Mutant polypeptide
MGKASYDNVDTLIEKGRYNTKYNYLKRMEKYAPNAMAYFDKVTINPQGNDFYINNPKVELDGEPSMNYLEDVYFGKALLTNDTQQEQKLKSQSFTCKNTDTVTATTTHTVGTSIQATAKFTVPFNETGVSLTTSYSFANTNTNTNSKEITHNVPSQDILVPANTTVEAIFYLKKVNVKGNVKLVGQVSGSEWGEIPSALAFPRDGYKFSLSDTVNKSDLNEDGTININGKGNYSAVMGDELIVKVRNLNTNNVQEYVIPVDKK

SEQ ID NO: 41 - protein, 263 aa, Artificial Sequence
  Mutant polypeptide
MGKASYDNVDTLIEKGRYNTKYNYLKRMEKYAPNAMAYFDKVTINPQGNDFYINNPKVELDGEPSMNYLEDVYVGKALLTNDTQQEQKLKSQSATCKNTDTVTATTTHTVGTSIQATAKFTVPFNETGVSLTTSYSFANTNTNTNSKEITHNVPSQDILVPANTTVEAIFYLKKVNVKGNVKLVGQVSGSEWGEIPSALAFPRDGYKFSLSDTVNKSDLNEDGTININGKGNYSAVMGDELIVKVRNLNTNNVQEYVIPVDKK

SEQ ID NO: 42 - protein, 263 aa, Artificial Sequence
  Mutant polypeptide
MGKASYDNVDTLIEKGRYNTKYNYLKRMEKYAPNAMAYFDKVTINPQGNDFYINNPKVELDGEPSMNYLEDVYFGKALLTNDTQQEQKLKSQSATCKNTDTVTATTTHTVGTSIQATAKFTVPFNETGVSLTTSYSFANTNTNTNSKEITANVPSQDILVPANTTVEAIAYLKKVNVKGNVKLVGQVSGSEWGEIPSALAFPRDGYKFSLSDTVNKSDLNEDGTININGKGNYSAVMGDELIVKVRNLNTNNVQEYVIPVDKK

SEQ ID NO: 43 - protein, 263 aa, Artificial Sequence
  Mutant polypeptide
MGKASYDNVDTLIEKGRYNTKYNYLKRMEKYAPNAMAYFDKVTINPQGNDFYINNPKVELDGEPSMNYLEDVYFGKALLTNDTQQEQKLKSQSATCKNTDTVTATTTHTVGTSIQATAKFTVPFNETGVSLTTSYSFANTNTNTNSKEITANVPSQDILVPANTTVEVIFYLKKVNVKGNVKLVGQVSGSEWGEIPSALAFPRDGYKFSLSDTVNKSDLNEDGTININGKGNYSAVMGDELIVKVRNLNTNNVQEYVIPVDKK

SEQ ID NO: 44 - protein, 263 aa, Artificial Sequence
  Mutant polypeptide
MGKASYDNVDTLIEKGRYNTKYNYLKRMEKYAPNAMAYFDKVTINPQGNDFYINNPKVELDGEPSMNYLEDVYFGKALLTNDTQQEQKLKSQSATCKNTDTVTATTTHTVGTSIQATAKFTVPFNETGVSLTTSYSFANTNTNTNSKEITHNVPSQDILVPANTTVEAIFYLKKVNVKGNVKLVGQVSGSEWGEIPSALAFPRDGYKFSLSDTVNKSDLNEDGTININGKGNYSAVMGDELIVKVRNLNTNNVQEYVIPVDKK

SEQ ID NO: 45 - protein, 263 aa, Artificial Sequence
  Mutant polypeptide
MGKASYDNVDTLIEKGRYNTKYNYLKRMEKYAPNAMAYFDKVTINPQGNDFYINNPKVELDGEPSMNYLEDVYFGKALLTNDTQQEQKLKSQSATCKNTDTVTATTTHTVGTSIQATAKFTVPFNETGVSLTTSYSFANTNTNTNSKEITANVPSQDILVPANTTVEAIFYLKKVNVKGNVKLVGQVSGSEWGEIPSALAFPRDGYKFSLSDTVNKSDLNEDGTININGKGNYSAVMGDELIVKVRNLNTNNVQEYVIPVDKK

SEQ ID NO: 46 - protein, 263 aa, Artificial Sequence
  Mutant polypeptide
MGKASYDNVDTLIEKGRYNTKYNYLKRMEKYYPNAMAYFDKVTINPQGNDFYINNPKVELDGEPSMNYLEDVYFGKALLTNDTQQEQKLKSQSFTCKNTDTVTATTTHTVGTSIQATAKFTVPFNETGVSLTTSYSFANTNTNTNSKEITHNVPSQDILVPANTTVEVIAYLKKVNVKGNVKLVGQVSGSEWGEIPSYLAFPRDGYKFSLSDTVNKSDLNEDGTININGKGNYSAVMGDELIVKVRNLNTNNVQEYVIPVDKK

SEQ ID NO: 47 - protein, 263 aa, Artificial Sequence
  Mutant polypeptide
MGKASYDNVDTLIEKGRYNTKYNYLKRMEKYYPNAMAYFDKVTINPQGNDFYINNPKVELDGEPSMNYLEDVYVGKALLTNDTQQEQKLKSQSATCKNTDTVTATTTHTVGTSIQATAKFTVPFNETGVSLTTSYSFANTNTNTNSKEITHNVPSQDILVPANTTVEVIAYLKKVNVKGNVKLVGQVSGSEWGEIPSYLAFPRDGYKFSLSDTVNKSDLNEDGTININGKGNYSAVMGDELIVKVRNLNTNNVQEYVIPVDKK

SEQ ID NO: 48 - protein, 263 aa, Artificial Sequence; identical to SEQ ID NO: 14
  Mutant polypeptide

SEQ ID NO: 49 - protein, 263 aa, Artificial Sequence
  Mutant polypeptide
MGKASYDNVDTLIEKGRYNTKYNYLKRMEKYYPNAMAYFDKVTINPQGNDFYINNPKVELDGEPSMNYLEDVYVGKALLTNDTQQEQKLKSQSFTCKNTDTVTATTTHTVGTSIQATAKFTVPFNETGVSLTTSYSFANTNTNTNSKEITHNVPSQDILVPANTTVEAIAYLKKVNVKGNVKLVGQVSGSEWGEIPSYLAFPRDGYKFSLSDTVNKSDLNEDGTININGKGNYSAVMGDELIVKVRNLNTNNVQEYVIPVDKK

SEQ ID NO: 50 - protein, 263 aa, Artificial Sequence
  Mutant polypeptide
MGKASYDNVDTLIEKGRYNTKYNYLKRMEKYYPNAMAYFDKVTINPQGNDFYINNPKVELDGEPSMNYLEDVYVGKALLTNDTQQEQKLKSQSFTCKNTDTVTATTTHTVGTSIQATAKFTVPFNETGVSLTTSYSFANTNTNTNSKEITHNVPSQDILVPANTTVEVIFYLKKVNVKGNVKLVGQVSGSEWGEIPSYLAFPRDGYKFSLSDTVNKSDLNEDGTININGKGNYSAVMGDELIVKVRNLNTNNVQEYVIPVDKK

SEQ ID NO: 51 - DNA, 83 bp, Artificial Sequence
  Primer sequence
gaaaggaagatataatacaaaatataattacttaaagagaatggaaaaatatgcgcctaatgctatggcatattttgataagg

SEQ ID NO: 52 - DNA, 83 bp, Artificial Sequence
  Primer sequence
ccttatcaaaatatgccatagcattaggcgcatatttttccattctctttaagtaattatattttgtattatatcttcctttc

SEQ ID NO: 53 - DNA, 49 bp, Artificial Sequence
  Primer sequence
gtgaatggggagagatacctagtgcgttagcttttcctagggatggtta

SEQ ID NO: 54 - DNA, 49 bp, Artificial Sequence
  Primer sequence
taaccatccctaggaaaagctaacgcactaggtatctctccccattcac

SEQ ID NO: 55 - DNA, 65 bp, Artificial Sequence
  Primer sequence
caaatacaaatacaaatactaattcaaaagaaattactgctaatgtcccttcacaagatatacta

SEQ ID NO: 56 - DNA, 65 bp, Artificial Sequence
  Primer sequence
tagtatatcttgtgaagggacattagcagtaatttcttttgaattagtatttgtatttgtatttg

SEQ ID NO: 57 - DNA, 54 bp, Artificial Sequence
  Primer sequence
agaaccatcaatgaattatcttgaagatgtttattttggaaaagctctcttaac

SEQ ID NO: 58 - DNA, 54 bp, Artificial Sequence
  Primer sequence
gttaagagagcttttccaaaataaacatcttcaagataattcattgatggttct

SEQ ID NO: 59 - DNA, 76 bp, Artificial Sequence
  Primer sequence
tcttaactaatgatactcaacaagaacaaaaattaaaatcacaatcagcgacttgtaaaaatactgatacagtaac

SEQ ID NO: 60 - DNA, 76 bp, Artificial Sequence
  Primer sequence
gttactgtatcagtatttttacaagtcgctgattgtgattttaatttttgttcttgttgagtatcattagttaaga

SEQ ID NO: 61 - DNA, 64 bp, Artificial Sequence
  Primer sequence
atactagtaccagctaatactactgtagaagcgatagcatatttaaaaaaagttaatgttaaag

SEQ ID NO: 62 - DNA, 64 bp, Artificial Sequence
  Primer sequence
ctttaacattaactttttttaaatatgctatcgcttctacagtagtattagctggtactagtat

SEQ ID NO: 63 - DNA, 82 bp, Artificial Sequence
  Primer sequence
gatatactagtaccagctaatactactgtagaagtaatattttatttaaaaaaagttaatgttaaaggaaatgtaaagttag

SEQ ID NO: 64 - DNA, 82 bp, Artificial Sequence
  Primer sequence
ctaactttacatttcctttaacattaactttttttaaataaaatattacttctacagtagtattagctggtactagtatatc

SEQ ID NO: 65 - protein, 260 aa, Artificial Sequence
  Protein fragment
KASYDNVDTLIEKGRYNTKYNYLKRMEKYYPNAMAYFDKVTINPQGNDFYINNPKVELDGEPSMNYLEDVYVGKALLTNDTQQEQKLKSQSFTCKNTDTVTATTTHTVGTSIQATAKFTVPFNETGVSLTTSYSFANTNTNTNSKEITHNVPSQDILVPANTTVEVIAYLKKVNVKGNVKLVGQVSGSEWGEIPSYLAFPRDGYKFSLSDTVNKSDLNEDGTININGKGNYSAVMGDELIVKVRNLNTNNVQEYVIPVDK

SEQ ID NO: 66 - protein, 32 aa, Artificial Sequence
  Protein fragment
MKKNLVKSLAIASAVISIYSIVNIVSPTNVIA

SEQ ID NO: 67 - protein, 13 aa, Artificial Sequence
  Protein fragment
KEISNTVSNEMSK

SEQ ID NO: 68 - protein, 23 aa, Artificial Sequence
  Protein fragment
KEKSNDSNIVKYRSLYIKAPGIK